European Patent Application EP 4 640 826 A1, published October 29, 2025. Title: A novel L-ligase and preparation method of L-carnosine using the same. Applicant: CJ CheilJedang Corporation. The sequence listing filed with the application follows.

SEQUENCE LISTING (58 sequences)

SEQ ID NO: 1 - protein, 472 aa, Bacillus subtilis
MERKTVLVIADLGGCPPHMFYKSAAEKYNLVSFIPRPFAITASHAALIEKYSVAVIKDKDYFKSLADFEHPDSIYWAHEDHNKPEEEVVEQIVKVAEMFGADAITTNNELFIAPMAKACERLGLRGAGVQAAENARDKNKMRDAFNKAGVKSIKNKRVTTLEDFRAALEEIGTPLILKPTYLASSIGVTLITDTETAEDEFNRVNDYLKSINVPKAVTFEAPFIAEEFLQGEYGDWYQTEGYSDYISIEGIMADGEYFPIAIHDKTPQIGFTETSHITPSILDEEAKKKIVEAAKKANEGLGLQNCATHTEIKLMKNREPGLIESAARFAGWNMIPNIKKVFGLDMAQLLLDVLCFGKDADLPDGLLDQEPYYVADCHLYPQHFKQNGQIPETAEDLVIEAIDIPDGLLKGDTEIVSFSAAAPGTSVDLTLFEAFNSIAAFELKGSNSQDVAESIRQIQQHAKLTAKYVLPV

SEQ ID NO: 2 - protein, 473 aa, Streptococcus pneumoniae
MSKKTVLVIADLGGCPPHMFYESVAASYHIVSYIPRPFAITKGHAELIEKYSIAVIKDRDYFETHPSFEHPDSIYWAHDDYPKSEEEVVEDFIRVASFFKADAITTNNELFIAPMAKAAERLGLRGAGVKAAEMARDKSQMRAAFNASGVKAVKTQPVTTLSDFQKAIESIGTPLILKPTYLASSIGVTLFHDKAGSDDLFLQVQSYLETIPVPDAVTYEAPFVAETYLEGAYEDWYEDEGYADYVSVEGLVVEGEYLPFVIHDKTPQIGFTETAHITPTILDNEAKQIIIEAARKANEGLGLEHCATHTEIKLMKNRETGLIESAARFAGWNMIPNIKKVFGVDMAKLLIDVLVDGKKAVLPKQLLSGHTFYVADCHLYPQHFKESGHIPPESTHITIDHVSIPQEAFVGDTAIVSQSFPTKGTIVDLELFEAFNGIVSLELKGSSSQDVAASIRNIQKQATIQLMDELVKG

SEQ ID NO: 3 - protein, 472 aa, Alkalihalobacillus halodurans
MERKTVLVIADLGGCPPHMFYQSAAEKYNLVSFIPRPFAITASHAALIEKYSVAVIKDKDYFQSITDFEHPDSIYWAHEDHDKPEEEVVEQIVKVAEMFGAEAITTNNELFIAPMAKACKRLGLRGAGVQAAENARDKNKMRAAFNKAGVKTIKNKRVTTLEDFRSALKEIGTPLILKPTYLASSIGVTLITDTKTAEAEFNRVNDYLKSINVPKAVTFEAPFIAEEFLQGEYPDWYQTEGYSDYISIEGIMADGEYFPVAIHDKTPQIGFTETSHITPSILDDEAKKIIIEAAKKANEGLGLENCATHTEIKLMKNREAGLIESAARFAGWNMIPNIKKVFGVDMAQLLLDVLCFGKDADLPDGLLEQEPCYIADCHLYPEHFKQNGQLPEAAEDMIIESINIPDGLLKGDTELVSFSAAAPGTSVDLRLFEAFNSIAAFELKGSNSQDVADSIKHIQQHAKLTAKYVLPV

SEQ ID NO: 4 - protein, 473 aa, Priestia megaterium
MKRKTVLVIADLGGCPPHMFYKSVAESYNIVSYIPRPFAITKSHANFIENYSVAVVKDVDYLKKISDFEHPDSIYWAQKEYDKPEEAVVEDIIKVATMFNVEAITTNNELFIAPMAKACEKLGLRGAGVEAAQKARDKNLMRESFNNSGVKAIKSKRVNTLKDFKEALEYVGVPLVLKPTYLASSIGVTFIYNEQDAEKIFLDAQEYLNSIGVPKAVTFEAPFIVEEFLQGEYEDWYTEPGYSDYVSVEGMMVGGKYYPLAIHDKTPQIGFTETAHITSTILDEDAKNKILDAVKKANEGLGLEHCATHTEVKLMKNREVGIIETAARFAGWNMIPNIKKSFNVDAAKVLVDILCEGYSEDLPKELLTDPYNYVADFHLYPHDFKTNGHLLENVSNIIFESIEIPENILVGDTKINSFNTVDKGTQLDLTLFEAFNGLAYLELHGTSSQDIVKSIQEIKKYAKLYLQGVPVTT

SEQ ID NO: 5 - protein, 419 aa, Pseudomonas syringae
MTQAKENILVVVDGYSSGSQLPTLMAESGWKCVHVSSSANPPEYYLRTYHKDEYIAHFEYQGDIQSLASAVEAWHPAAVLPGTESGVIVADLLAAALQLPGNDPSTSLARRDKYTMHESLKAVGLRSMDHFLAVDRDALSAWAERGSWPVVIKPQASAGTDSVTFCADQGELLESFDQLFGTVNQLGERNNAVLAQRLLVGPEYFINGVSGHGKHLITEIWRADKLPAPDGGWIYDRAVLFDPTSPEMQEIVRYVHGVLDALGIRYGANHTELIVTADGPTLIECASRLSGGLHRPAANYAVGASQLDLVGKLVREGESAIDDILQTWQPHRYALWQVQFISNQEGVVARSSYDELLKTLKSNAWLQRAPKEGDTVVKTVDLFSSPGIVFMSHADGNVLHDDYRTVREWERTSRLFSVQ

SEQ ID NO: 6 - protein, 414 aa, Pseudomonas syringae pv. phaseolicola
MKKIILIETSDVATRYSALAVLKLGFEPLFIIGSARYYQGDTFTQLMEFPYLECGDTTNVDAVLKLIGALPKDSIEAILSLVETRIPIAVELASTLGVKGLDCALARLGGKEYVSSLIPEYSPISMEVGEFSNFSMLVRGPFAHCKKVIVKPVRGSGAAGYAEFSLSDSEFNEKILAHIQSCALSLGAHEFIMQEYVDGELISLEGYAVAGQCHFLGVSLRRKIANTESVNYFPASKYFTEEVIQRAKLAVEAIVLRSGLQQGYFHSEFKIGPKTAVLIDANFGRVAGAAISEQIALSYQCDPVYFFKHVIEVGCLQSEATLNVSSPIDTISIFYGLPVQARINDIKFSLDWSLNHTRVLDIFTSVDPMGRDDWGWIALVSGRAQDVRRQIDGLLIVTDKGTYTPFYIDSSEPL

SEQ ID NO: 7 - protein, 477 aa, Bacillus pumilus
MVLSLSKKTVLVIADLGGCPPHMFYESVAASYHIVSYIPRPFAITKGHAELIEKYSIAVIKDRDYFETHPSFEHPDSIYWAHDDYPKSEEEVVEDFIRVASFFKADAITTNNELFIAPMAKAAERLGLRGAGVKAAEMARDKSQMRAAFNASGVKAVKTQPVTTLSDFQQAIESIGTPLILKPTYLASSIGVTLFHDKAGSDDLFLQVQSYLETIPVPDAVTYEAPFVAETYLEGAYEDWYEDEGYADYVSVEGLVVEGEYLPFVIHDKTPQIGFTETAHITPTILDNEAKQIIIEAARKANEGLGLEHCATHTEIKLMKNRETGLIEAAARFAGWNMIPNIKKVFGVDMAKLLIDVLVDGKKAVLPKQLLSGHTFYVADCHLYPQHFKESGLIPPEATHITIDHVSIPQEAFVGDTAIVSQSFPAKGTIVDLELFEAFNGIVSLELKGSSSQDVAASIRNIQKQATIQLMDELVKG

SEQ ID NO: 8 - protein, 473 aa, synthetic construct
MSKKTVLVIADLGGCPPHMFYESVAASYHIVSYIPRPFAITKGHAELIEKYSIAVIKDRDYFETHPSFEHPDSIYWAHDDYPKSEEEVVEDFIRVASFFKADAITTNEELFIAPMAKAAERLGLRGAGVKAAEMARDKSQMRAAFNASGVKAVKTQPVTTLSDFQKAIESIGTPLILKPTYLASSIGVTLFHDKAGSDDLFLQVQSYLETIPVPDAVTYEAPFVAETYLEGAYEDWYEDEGYADYVSVEGLVVEGEYLPFVIHDKTPQIGFTETAHITPTILDNEAKQIIIEAARKANEGLGLEHCATHTEIKLMKNRETGLIESAARFAGWNMIPNIKKVFGVDMAKLLIDVLVDGKKAVLPKQLLSGHTFYVADCKLYPQHFKESGHIPPESTHITIDHVSIPQEAFVGDTAIVSQSFPTKGTIVDLELFEAFNGIVSLELKGSSSQDVAASIRNIQKQATIQLMDELVKG

SEQ ID NO: 9 - protein, 136 aa, Corynebacterium glutamicum
MLRTILGSKIHRATVTQADLDYVGSVTIDADLVHAAGLIEGEKVAIVDITNGARLETYVIVGDAGTGNICINGAAAHLINPGDLVIIMSYLQATDAEAKAYEPKIVHVDADNRIVALGNDLAEALPGSGLLTSRSI

SEQ ID NO: 10 - DNA, 1419 bp, Bacillus subtilis
  source 1..1419: mol_type = genomic DNA
atggagcgtaaaacggtgctggtgatcgctgacctgggcggctgtcctccccacatgttctacaaatccgctgcagaaaagtacaatctcgtgtccttcattccgcgccccttcgcgattacggcttcccatgccgcactcattgaaaagtacagcgtggcagtgattaaggataaagattattttaaatccctggcggacttcgaacatccggactcaatctattgggctcacgaggaccacaataagcctgaagaggaagtggtcgagcaaattgttaaggtggcggagatgtttggagctgatgcaatcacgactaataatgagctgttcatcgctccgatggcaaaagcatgtgaacggcttggacttcgcggagcaggcgtccaagctgctgagaacgctcgggataaaaataaaatgcgtgacgcattcaataaggcaggagtgaagagcatcaagaacaaacgcgttaccacgctcgaagattttcgggcagccctggaagaaattggcacgccactcatcttgaaacctacttatctggcttcttcaattggagtgacccttattacggatacggaaactgcagaggatgaatttaaccgggttaacgactatctcaaatcaattaacgtgcccaaggctgtgacgttcgaagctcctttcatcgctgaggagttcttgcaaggagaatacggtgattggtaccaaacggagggatattctgattatatttcaattgaaggaatcatggccgatggagagtatttcccaattgcaattcacgataaaacgccacaaatcggattcaccgagactagccatatcacgccctcgatcctggacgaagaagccaaaaagaaaattgttgaggcggctaaaaaagcaaacgagggacttggactgcaaaactgcgctacccatacggaaatcaaactgatgaaaaaccgcgagccaggccttatcgaatccgcggctcgttttgctggttggaacatgatccctaacattaaaaaggtcttcggtcttgatatggcgcaattgttgttggacgttctctgctttggtaaagatgccgacttgccggatggtcttttggaccaagaaccctactacgtcgcggactgccatttgtatccccaacattttaaacaaaacggacaaattccggaaactgcagaagacttggtcatcgaggctatcgatattccagatggtctccttaaaggtgatactgagattgtgtcctttagcgcggctgcaccaggcactagcgtagatttgaccctgtttgaagcattcaatagcatcgccgcattcgagctgaagggatcaaattcacaggatgttgcggagagcattcgccagatccagcaacatgcaaagcttactgcgaaatatgtcctcccggtgtga

SEQ ID NO: 11 - DNA, 1422 bp, Streptococcus pneumoniae
  source 1..1422: mol_type = genomic DNA
atgagcaagaagactgttcttgtcatcgcggatttgggaggctgcccacctcatatgttctacgagagcgtcgcggcatcttaccatatcgtatcatatattccccgtccattcgccattaccaagggtcacgcagagctcattgagaaatattcgattgcagtcattaaagaccgtgattacttcgagacgcatccgtcgttcgaacatcccgattcgatctattgggcacacgatgattatcctaaatcggaagaagaagtagtcgaagacttcattcgtgttgcaagctttttcaaggccgatgcgattacgacgaacaatgaactgtttattgccccaatggcgaaggcagctgagcgtttgggattgcgcggagctggcgttaaggccgctgaaatggcccgtgataaatcccaaatgcgggccgcatttaatgcgtcaggcgttaaagctgtcaagacgcaaccggtgacgaccctctcagactttcagaaggctattgagtcaatcggtacgccgttgattctcaagccaacctatttggcatcctcaatcggcgtgacgcttttccacgacaaggctggctctgacgacctttttctgcaggttcagtcttatcttgaaactatcccagtacctgatgctgttacttacgaagcgccttttgtagccgagacttatctcgagggtgcctatgaggactggtatgaggacgaaggttatgccgactacgtgtcagttgagggactcgttgtcgaaggtgaatatctccccttcgttattcacgacaagacgcctcagattggttttaccgagacggcccacattaccccgactatcctggacaacgaagcgaagcagatcatcatcgaagccgcccggaaagctaatgagggtcttggtcttgagcactgcgcgactcataccgagattaaactgatgaagaatcgggagaccggactgatcgaatccgcagctcgctttgccggatggaacatgattcccaacatcaagaaagtgttcggtgtggacatggcgaaacttctcatcgatgtactcgttgacggtaagaaggcagtacttccgaagcagttgctgagcggccacacgttttatgtggcagattgtcatctttatcctcaacattttaaagaatcgggccacatccctccagagtcgacgcatattaccattgaccacgtgtctatccctcaagaggcgttcgtcggcgatacggcgattgtatcacagtcatttcccacgaagggaacgattgtagatctggagctcttcgaagccttcaacggaatcgtgtccttggaactgaagggctcgtcttcgcaggatgttgccgcctctatccgtaacatccagaaacaagccacgatccaacttatggacgagcttgtgaagggctaa

SEQ ID NO: 12 - DNA, 1419 bp, Alkalihalobacillus halodurans
  source 1..1419: mol_type = genomic DNA
atggaacgtaagactgtactggtcatcgcggacctgggaggctgtccgccacacatgttttaccagtccgcggccgagaagtacaaccttgtgagctttattcctcgtccgttcgctattactgcgtcacacgccgcgctcatcgaaaaatactccgtggcggtaattaaggacaaggactacttccagtcaattaccgatttcgagcaccccgactcgatttactgggcccatgaagaccacgataaaccggaggaagaagtggttgaacagattgtaaaagtggctgagatgtttggtgctgaagctatcactaccaacaatgagctcttcatcgcccctatggcaaaggcctgcaaacggctcggtctccggggagcgggcgttcaagcggccgaaaatgctcgcgacaaaaataaaatgcgggctgctttcaataaggctggtgtgaagaccattaagaataagcgggtaaccacgctggaagactttcgctcagcactgaaagaaatcggtacgccgttgattttgaagcctacctatctcgcgagctcaattggagtcacgctcatcaccgacaccaagactgcagaggcagaatttaaccgtgtcaacgactacctgaagtcgatcaatgtccccaaggccgtcaccttcgaagcgccgttcattgccgaggagttcctgcagggagaatatccagactggtatcagactgagggttattctgactatatttcaattgaaggtatcatggccgacggtgagtactttcccgtggcaattcacgacaaaaccccccagatcggatttaccgagacctcgcacatcactccgtccatcctggatgacgaagcaaaaaagattattatcgaagccgctaaaaaagccaacgagggacttggccttgaaaattgcgcgactcataccgaaattaagcttatgaagaaccgtgaagcgggtcttattgaatcagccgctcgtttcgcaggatggaacatgatcccaaacatcaaaaaggtgtttggtgttgacatggcacaacttttgctggatgtactgtgcttcggaaaggacgctgaccttccggatggtctcctcgaacaggagccgtgctatatcgccgactgccatctttacccggaacatttcaagcaaaacggtcaactccctgaagccgcagaggacatgatcatcgaatctattaatatccctgacggcttgctcaagggcgacacggaattggtctcgttcagcgcggctgcgccgggaactagcgttgaccttcgcctctttgaggcttttaattcaattgcggcattcgaactgaagggtagcaactcccaggatgttgcagactctattaagcacattcaacaacacgctaagctgaccgcaaagtacgttctgccggtctaa

SEQ ID NO: 13 - DNA, 1422 bp, Priestia megaterium
  source 1..1422: mol_type = genomic DNA
atgaagcgtaagactgttctggttattgcagacctcggaggttgccctccacatatgttctacaagtcggtggcggagtcttataatatcgtatcgtatattccacggccttttgcgatcactaaatcgcacgctaatttcatcgaaaactattcagtggccgtcgtcaaggatgtggattacctgaaaaagatctcggactttgaacacccagactcgatctattgggcacaaaaagaatatgacaaaccggaggaagcggtagtcgaggatattattaaggtagcaacgatgtttaacgtggaagcaattaccaccaataatgagcttttcattgccccaatggctaaggcatgcgaaaagttgggtctccggggcgcgggtgtcgaggcggcccagaaggcgcgtgacaaaaatttgatgcgcgaatcatttaataactctggtgttaaagccatcaaatctaagcgggttaacacgctgaaggatttcaaagaggccctcgaatacgtcggtgttcctcttgtgctcaaaccgacctatcttgcgtcgtcaatcggtgtcaccttcatctacaatgagcaagatgccgaaaaaatcttcctggatgctcaggaatatttgaattccattggcgtgcccaaggctgtgactttcgaggcaccattcattgtagaagagtttcttcagggtgaatatgaggactggtatacggagccgggctatagcgactacgtctccgttgagggtatgatggtgggcggaaagtattaccctttggctatccacgacaaaacgcctcagatcggctttactgagacggctcatattacttctactatcctcgatgaagacgctaagaataaaattttggatgctgtaaagaaggctaatgaaggtttgggacttgaacattgtgctactcacactgaggtcaaattgatgaagaaccgcgaggtcggaattattgaaactgccgcacggtttgcaggctggaacatgattcctaatattaagaagtcctttaacgtcgatgccgctaaagtcctggtggatatcctttgtgaaggatactccgaagacctccccaaagaacttctgaccgatccatacaactatgttgctgatttccatttgtatccacatgacttcaaaaccaatggtcatctcctcgaaaacgtctctaatattattttcgagagcatcgaaatccccgagaacatcctcgttggagacactaagatcaactcgtttaacaccgtagataagggaacgcagttggatctcacgctctttgaagctttcaatggcctcgcctaccttgaactgcacggtacgtcatcccaggacattgtcaagtccattcaggaaatcaagaaatatgcgaaactttacctgcagggcgtgcctgtgactacgtaa

SEQ ID NO: 14 - DNA, 1260 bp, Pseudomonas syringae
  source 1..1260: mol_type = genomic DNA
atgacgcaggcaaaagagaatattctggtcgtggtagatggctactcctccggatcacaactccccacccttatggctgaatccggctggaaatgtgtccatgtaagctcaagcgcaaatccgccagaatactatctccgcacttatcacaaggacgaatacatcgcacactttgaataccaaggagacatccagtctctcgcttctgccgtcgaggcctggcacccagccgcggtgctccctggtactgagtcaggcgttatcgtcgccgatttgttggccgcagcactccagttgccaggaaatgatccatccacttccctcgcacgccgtgataaatacaccatgcacgaaagcctgaaagctgtaggtcttcgttcaatggaccactttcttgcagtagatcgtgatgcactttccgcatgggcggaacgcggttcttggcctgtggttatcaagccgcaggcctcggccggtactgactccgtaacgttctgtgctgaccaaggtgagctgcttgaatcttttgaccaactctttggcacggttaaccaacttggcgaacgtaataatgccgttttggcacaacgcctgctggtcggcccggaatatttcattaatggcgtctcgggccacggcaaacatctcattactgaaatttggcgcgctgacaagctgcctgcccctgatggtggttggatctatgatcgtgcggtgctgttcgatcccacttcgccagaaatgcaggagatcgttcggtacgtccacggcgttttggatgcattgggaatccgttatggagcaaatcacacggagctcatcgttacggcagacggacccactctcatcgagtgcgcctcacggctttcgggtggactgcatcgcccagctgcgaactacgctgtcggtgcatcgcagctcgatttggttggaaagttggtacgtgagggtgaatccgccattgacgatattcttcagacgtggcagcctcatcgttatgccctttggcaagtgcaatttatctctaaccaggaaggcgtagtggctcgctcgtcctatgatgaactcttgaaaactcttaaatccaacgcctggctccagcgcgctcctaaagaaggtgatactgttgtaaagacggtcgatttgttctcgagccctggaattgtgttcatgtctcatgcagatggcaatgttctgcatgatgactatcggactgttcgtgaatgggagcgtacttcacggctcttttccgtccagtaa

SEQ ID NO: 15 - DNA, 1245 bp, Pseudomonas syringae pv. phaseolicola
  source 1..1245: mol_type = genomic DNA
atgaaaaagattattctcattgaaacctcagatgttgccacccgttacagcgcactcgctgtgttgaaactcggtttcgaacctctgttcatcatcggctccgcacgttactatcaaggtgatacttttacgcagctcatggaattcccttatctggaatgcggtgacaccacgaacgtcgatgccgtgttgaagctgatcggtgcattgcccaaagactcaatcgaggctattctgtctcttgtggaaacgcgtatcccaatcgccgtcgaacttgcttccactcttggcgttaaaggcctggactgcgcactcgcgcgtcttggcggaaaggaatatgtatcgtctctcatccctgagtattctccgatttcgatggaagtcggcgagttctcaaacttctctatgctcgtacgtggtccgtttgcacattgcaaaaaggttatcgtgaagccagtgcgtggctcaggagcggctggctatgctgaatttagcctttcggatagcgagtttaatgagaaaatcctcgcacatattcagtcttgtgcactgtctctcggtgcccatgaattcattatgcaggagtacgtggatggcgagttgatttccctcgaaggttacgcagtcgccggtcagtgccactttttgggcgtctccctccgccgcaaaatcgcgaacaccgaatcggtgaactattttcccgcatcaaaatattttacggaggaagtcatccaacgcgctaagttggcagtggaggctattgttttgcgctcgggtctccagcagggctacttccatagcgaattcaagatcggtccgaagactgccgttctcatcgacgccaacttcggacgggtcgctggtgctgctatttcagaacagattgcgctgtcctatcagtgtgatcccgtatacttcttcaagcatgtaatcgaggttggatgtttgcaaagcgaagcgaccttgaatgtaagctctccgatcgatactattagcatcttctacggcctcccggttcaagctcgtattaatgatattaagttcagcttggattggtcgttgaatcatactcgggtcttggacatttttacctctgttgatccgatgggtcgtgacgattggggatggattgcacttgtttctggtcgcgcccaggatgttcgtcgccaaattgatggccttcttattgttacggataaaggtacctatacgccattctacatcgattcgtcagaacctctttaa

SEQ ID NO: 16 - DNA, 1434 bp, Bacillus pumilus
  source 1..1434: mol_type = genomic DNA
atggtccttagcctgtcgaaaaagaccgtattggtaattgcagatctgggaggttgcccgccgcatatgttttacgagtctgtagcggcttcctaccacatcgtgtcttacatcccgcgcccctttgccattactaagggacatgcggaactcatcgagaaatattctattgcggtgattaaagaccgcgactattttgagacccatccctcgttcgagcatcccgactctatctactgggcgcacgacgattacccgaagagcgaggaggaagtcgtggaagattttattcgggtagcgtcttttttcaaagctgacgctattacgacgaataatgaactgtttatcgcgccgatggcaaaggcagccgagcgtcttggtttgcgtggagcgggtgttaaagcggcagaaatggcgcgcgataagtcacaaatgcgggcggcattcaacgcatccggcgttaaggcagtgaagactcaacctgttactacgttgagcgactttcagcaagcaattgagagcattggcactccgttgattcttaagcctacttatttggcatcgtctattggcgtgactctgtttcatgacaaagcaggttcggatgacctttttctgcaggttcaatcttatcttgaaactatcccagtgccagacgcggtcacctacgaggccccattcgttgccgaaacctatctcgaaggagcttatgaggattggtacgaagatgaaggatacgccgactatgttagcgtagagggcctggtagtagaaggcgagtatttgccatttgtgatccacgacaaaacccctcagattggctttacggagaccgcgcacatcactcccacgattctcgacaacgaagcaaagcaaattattatcgaagctgcccggaaagcaaatgaaggtctcggcctcgagcattgcgcgactcacaccgagatcaagctgatgaaaaatcgcgagactggattgattgaagcggcagctcgtttcgctggatggaacatgattcctaatattaagaaagtctttggtgttgacatggctaagcttctgatcgacgtgttggtagatggtaagaaagccgtactccctaaacagttgttgtcgggtcacacgttttatgtagcagactgccacctgtatccgcagcatttcaaggagtcaggtctcatccccccggaggccacgcacatcacgattgatcacgtttcaatccctcaggaggcatttgtgggcgataccgcaatcgttagccagagcttcccagctaaaggtactatcgtggatttggaactctttgaggcgtttaacggtattgtatccctggaacttaagggaagctcaagccaagatgtcgctgcttctattcggaacatccaaaagcaggccaccattcaacttatggatgagttggtgaaaggttga

SEQ ID NO: 17 - DNA, 1422 bp, synthetic construct
  source 1..1422: mol_type = other DNA
atgagcaagaagactgttcttgtcatcgcggatttgggaggctgcccacctcatatgttctacgagagcgtcgcggcatcttaccatatcgtatcatatattccccgtccattcgccattaccaagggtcacgcagagctcattgagaaatattcgattgcagtcattaaagaccgtgattacttcgagacgcatccgtcgttcgaacatcccgattcgatctattgggcacacgatgattatcctaaatcggaagaagaagtagtcgaagacttcattcgtgttgcaagctttttcaaggccgatgcgattacgacgaacgaagaactgtttattgccccaatggcgaaggcagctgagcgtttgggattgcgcggagctggcgttaaggccgctgaaatggcccgtgataaatcccaaatgcgggccgcatttaatgcgtcaggcgttaaagctgtcaagacgcaaccggtgacgaccctctcagactttcagaaggctattgagtcaatcggtacgccgttgattctcaagccaacctatttggcatcctcaatcggcgtgacgcttttccacgacaaggctggctctgacgacctttttctgcaggttcagtcttatcttgaaactatcccagtacctgatgctgttacttacgaagcgccttttgtagccgagacttatctcgagggtgcctatgaggactggtatgaggacgaaggttatgccgactacgtgtcagttgagggactcgttgtcgaaggtgaatatctccccttcgttattcacgacaagacgcctcagattggttttaccgagacggcccacattaccccgactatcctggacaacgaagcgaagcagatcatcatcgaagccgcccggaaagctaatgagggtcttggtcttgagcactgcgcgactcataccgagattaaactgatgaagaatcgggagaccggactgatcgaatccgcagctcgctttgccggatggaacatgattcccaacatcaagaaagtgttcggtgtggacatggcgaaacttctcatcgatgtactcgttgacggtaagaaggcagtacttccgaagcagttgctgagcggccacacgttttatgtggcagattgtaaactttatcctcaacattttaaagaatcgggccacatccctccagagtcgacgcatattaccattgaccacgtgtctatccctcaagaggcgttcgtcggcgatacggcgattgtatcacagtcatttcccacgaagggaacgattgtagatctggagctcttcgaagccttcaacggaatcgtgtccttggaactgaagggctcgtcttcgcaggatgttgccgcctctatccgtaacatccagaaacaagccacgatccaacttatggacgagcttgtgaagggctaa

SEQ ID NO: 18 - DNA, 411 bp, synthetic construct
  source 1..411: mol_type = other DNA
atgctgcgcaccatcctcggaagtaagattcaccgagccactgtcactcaagctgatctagattatgttggctctgtaaccatcgacgccgacctggttcacgccgccggattgatcgaaggcgaaaaagttgccatcgtagacatcaccaacggcgctcgtctggaaacttatgtcattgtgggcgacgccggaacgggcaatatttgcatcaatggtgccgctgcacaccttattaatcctggcgatcttgtgatcatcatgagctaccttcaggcaactgatgcggaagccaaggcgtatgagccaaagattgtgcacgtggacgccgacaaccgcatcgttgcgctcggcaacgatcttgcggaagcactacctggatccgggcttttgacgtcgagaagcatttag

SEQ ID NO: 19 - protein, 463 aa, synthetic construct
MAKSNEGLGTGLRTRHLTMMGLGSAIGAGLFLGTGVGIRAAGPAVLLAYIIAGAIVVLVMQMLGEMAAARPASGSFSRYGEDAFGHWAGFSLGWLYWFMLIMVMGAEMTGAAAIMGAWFGVEPWIPSLVCVVFFAVVNLVAVRGFGEFEYWFAFIKVAVIIAFLIIGIALIFGWLPGSTFVGTSNFIGDHGFMPNGISGVAAGLLAVAFAFGGIEIVTIAAAESDKPREAISLAVRAVIWRISVFYLGSVLVITFLMPYESINGADTAAESPFTQILAMANIPGTVGFMEAIIVLALLSAFNAQIYATSRLVFSMANRQDAPRVFSKLSTSHVPTNAVLLSMFFAFVSVGLQYWNPAGLLDFLLNAVGGCLIVVWAMITLSQLKLRKELQANDEISTVRMWAHPWLGILTLVLLAGLVALMLGDAASRSQVYSVAIVYGFLVLLSFVTVNSPLRGGRTPSDLN

SEQ ID NO: 20 - DNA, 1392 bp, synthetic construct
  source 1..1392: mol_type = other DNA
atggctaaatctaatgaagggctgggaaccggacttcggacccgccacctcacaatgatgggactcggctccgcaattggtgccggactgttcctcggcaccggcgttggtatccgcgcagccggccccgcagtgctcctggcgtacatcatcgccggagccatcgttgtgcttgttatgcaaatgctcggcgagatggctgctgcccgtcccgcctccggatcgttttcacgttacggcgaggatgctttcggccactgggctggtttctccctcggttggttgtactggttcatgctgattatggtgatgggcgccgaaatgactggcgctgctgccatcatgggtgcatggttcggcgtcgaaccgtggattccttcgcttgtctgcgtggtcttcttcgctgtggtgaacctcgtcgcggttcgcggtttcggtgaattcgagtactggttcgcattcattaaggtcgcggtgatcatcgctttcctcatcattggtattgctcttattttcggatggcttcccggatccacctttgttggaacctcaaacttcatcggtgatcacggattcatgcccaatggtatttctggtgttgctgctggtttgctcgcggtggcttttgcctttggtggcattgaaattgtcaccattgcagctgcagagtccgataagccacgtgaagctatttccctggcggtgcgtgccgtgatttggcgtatttcagtcttttacttgggctctgttttggtcatcactttcctcatgccttatgagtcgatcaatggtgccgacaccgctgcggaatcccccttcacccaaatcctggcgatggcaaacatccctggcacggttggtttcatggaagcgatcatcgttctagcactgctttccgctttcaacgcccaaatctatgccacttctcgtttggtattttccatggcgaatcgacaagacgctccgcgagttttcagtaagctcagcaccagccacgtccccaccaatgcggtgctgttgtccatgttcttcgccttcgtttcagttggtttgcagtactggaatccagccggtctgcttgatttcctcctcaacgctgttggcggttgtttgattgtggtgtgggcaatgatcactttgtcacagttgaaactccgcaaagaactgcaagcaaacgatgaaatctccacggttcgcatgtgggcgcacccatggttaggcatcctcaccttggttttgttggcaggactcgttgctctcatgctcggcgacgcagcctcccgcagccaggtttactcagtggcaattgtgtacggattcttggttcttttgtccttcgtcacagttaacagcccattgcgcggaggtcgcaccccttccgacttgaactga

SEQ ID NO: 21 - DNA, 36 bp, synthetic construct
  source 1..36: mol_type = other DNA
gaggagatcaaaacaatggagcgtaaaacggtgctg

SEQ ID NO: 22 - DNA, 41 bp, synthetic construct
  source 1..41: mol_type = other DNA
cggtggcggccgctctagatcacaccgggaggacatatttc

SEQ ID NO: 23 - DNA, 37 bp, synthetic construct
  source 1..37: mol_type = other DNA
gaggagatcaaaacaatgagcaagaagactgttcttg

SEQ ID NO: 24 - DNA, 41 bp, synthetic construct
  source 1..41: mol_type = other DNA
cgcggtggcggccgctctagattagcccttcacaagctcgt

SEQ ID NO: 25 - DNA, 37 bp, synthetic construct
  source 1..37: mol_type = other DNA
gaggagatcaaaacaatggaacgtaagactgtactgg

SEQ ID NO: 26 - DNA, 40 bp, synthetic construct
  source 1..40: mol_type = other DNA
gcggtggcggccgctctagattagaccggcagaacgtact

SEQ ID NO: 27 - DNA, 37 bp, synthetic construct
  source 1..37: mol_type = other DNA
gaggagatcaaaacaatgaagcgtaagactgttctgg

SEQ ID NO: 28 - DNA, 41 bp, synthetic construct
  source 1..41: mol_type = other DNA
cgcggtggcggccgctctagattacgtagtcacaggcacgc

SEQ ID NO: 29 - DNA, 37 bp, synthetic construct
  source 1..37: mol_type = other DNA
gaggagatcaaaacaatgacgcaggcaaaagagaata

SEQ ID NO: 30 - DNA, 41 bp, synthetic construct
  source 1..41: mol_type = other DNA
cgcggtggcggccgctctagattactggacggaaaagagcc

SEQ ID NO: 31 - DNA, 39 bp, synthetic construct
  source 1..39: mol_type = other DNA
gagatcaaaacaatgaaaaagattattctcattgaaacc

SEQ ID NO: 32 - DNA, 41 bp, synthetic construct
  source 1..41: mol_type = other DNA
cggtggcggccgctctagattaaagaggttctgacgaatcg

SEQ ID NO: 33 - DNA, 39 bp, synthetic construct
  source 1..39: mol_type = other DNA
gaggagatcaaaacaatggtccttagcctgtcgaaaaag

SEQ ID NO: 34 - DNA, 46 bp, synthetic construct
  source 1..46: mol_type = other DNA
cggtggcggccgctctagatcaacctttcaccaactcatccataag

SEQ ID NO: 35 - DNA, 42 bp, synthetic construct
  source 1..42: mol_type = other DNA
cctgcagcccgggggatcccaataatcgtgaattttggcagc

SEQ ID NO: 36 - DNA, 42 bp, synthetic construct
  source 1..42: mol_type = other DNA
ggcggccgctctagatgttttgatctcctccaataatctatg

SEQ ID NO: 37 - DNA, 35 bp, synthetic construct
  source 1..35: mol_type = other DNA
ggaggagatcaaaacaatgctgcgcaccatcctcg

SEQ ID NO: 38 - DNA, 41 bp, synthetic construct
  source 1..41: mol_type = other DNA
cgtagccttggaatccactaaatgcttctcgacgtcaaaag

SEQ ID NO: 39 - DNA, 38 bp, synthetic construct
  source 1..38: mol_type = other DNA
ggctcccgcggtgaacaataatcgtgaattttggcagc

SEQ ID NO: 40 - DNA, 39 bp, synthetic construct
  source 1..39: mol_type = other DNA
ggatggtgcgcagcattgttttgatctcctccaataatc

SEQ ID NO: 41 - DNA, 18 bp, synthetic construct
  source 1..18: mol_type = other DNA
cctgggctagcggtgtag

SEQ ID NO: 42 - DNA, 18 bp, synthetic construct
  source 1..18: mol_type = other DNA
ctgctcttaaatccgcgg

SEQ ID NO: 43 - DNA, 36 bp, synthetic construct
  source 1..36: mol_type = other DNA
cgattacgacgaacgaagaactgtttattgccccaa

SEQ ID NO: 44 - DNA, 36 bp, synthetic construct
  source 1..36: mol_type = other DNA
ttggggcaataaacagttcttcgttcgtcgtaatcg

SEQ ID NO: 45 - DNA, 53 bp, synthetic construct
  source 1..53: mol_type = other DNA
ccacacgttttatgtggcagattgtaaactttatcctcaacattttaaagaat

SEQ ID NO: 46 - DNA, 53 bp, synthetic construct
  source 1..53: mol_type = other DNA
attctttaaaatgttgaggataaagtttacaatctgccacataaaacgtgtgg

SEQ ID NO: 47 - DNA, 39 bp, synthetic construct
  source 1..39: mol_type = other DNA
ggtttacggttgatacgtatttgcactctacgtagctgg

SEQ ID NO: 48 - DNA, 39 bp, synthetic construct
  source 1..39: mol_type = other DNA
cttcattagatttagccatgcccataagcctagtacgtc

SEQ ID NO: 49 - DNA, 38 bp, synthetic construct
  source 1..38: mol_type = other DNA
gagctcggtacccggggatccgttccccctggagtccg

SEQ ID NO: 50 - DNA, 41 bp, synthetic construct
  source 1..41: mol_type = other DNA
ctacgtagagtgcaaatacgtatcaaccgtaaacccacatg

SEQ ID NO: 51 - DNA, 39 bp, synthetic construct
  source 1..39: mol_type = other DNA
gtactaggcttatgggcatggctaaatctaatgaagggc

SEQ ID NO: 52 - DNA, 40 bp, synthetic construct
  source 1..40: mol_type = other DNA
cctgcaggtcgactctagaccaatgatgaggaaagcgatg

SEQ ID NO: 53 - DNA, 42 bp, synthetic construct
  source 1..42: mol_type = other DNA
gggtttacggttgatacagaaacatcccagcgctactaatag

SEQ ID NO: 54 - DNA, 41 bp, synthetic construct
  source 1..41: mol_type = other DNA
cttcattagatttagccatagtgtttcctttcgttgggtac

SEQ ID NO: 55 - DNA, 41 bp, synthetic construct
  source 1..41: mol_type = other DNA
gtagcgctgggatgtttctgtatcaaccgtaaacccacatg

SEQ ID NO: 56 - DNA, 41 bp, synthetic construct
  source 1..41: mol_type = other DNA
cccaacgaaaggaaacactatggctaaatctaatgaagggc

SEQ ID NO: 57 - DNA, 18 bp, synthetic construct
  source 1..18: mol_type = other DNA
ctctgcggtcccgcggac

SEQ ID NO: 58 - DNA, 21 bp, synthetic construct
  source 1..21: mol_type = other DNA
cgtgatcaccgatgaagtttg